European Patent Specification EP 4 101 926 B1, published October 22, 2025. Title: Novel glyceraldehyde-3-phosphate dehydrogenase variant and a method for producing L-valine using the same. Applicant: CJ CheilJedang Corporation. The sequence listing filed with the application follows.

SEQUENCE LISTING (10 sequences)

SEQ ID NO: 1 - protein, 334 aa, Artificial Sequence
  glyceraldehyde-3-phosphate dehydrogenase variant
MTIRVGINGFGRIGRNFFRAVLERSDDLEVVAVNDLTDNKTLSTLLKFDSIMGRLGQEVEYDDDSITVGGKRIAVYAERDPKNLDWAAHNVDIVIESTGFFTDANAAKAHIEAGAKKVIISAPASNEDATFVYSVNHESYDPENHNVISGASCTTNCLAPMAKVLNDKFGIENGLMTTVHAYTGDQRLHDAPHRDLRRARAAAVNIVPTSTGAAKAVALVLPELKGKLDGYALRVPVITGSATDLTFNTKSEVTVESINAAIKEAAVGEFGETLAYSEEPLVSTDIVHDSHGSIFDAGLTKVSGNTVKVVSWYDNEWGYTCQLLRLTELVASKL

SEQ ID NO: 2 - DNA, 1005 bp, Artificial Sequence
  glyceraldehyde-3-phosphate dehydrogenase variant coding gene
atgaccattcgtgttggtattaacggatttggccgtatcggacgtaacttcttccgcgcagttctagagcgcagcgacgatctcgaggtagttgcagtcaacgacctcaccgacaacaagaccctttccacccttctcaagttcgactccatcatgggccgccttggccaggaagttgaatacgacgatgactccatcaccgttggtggcaagcgcatcgctgtttacgcagagcgcgatccaaagaacctggactgggctgcacacaacgttgacatcgtgatcgagtccaccggcttcttcaccgatgcaaacgcggctaaggctcacatcgaagcaggtgccaagaaggtcatcatctccgcaccagcaagcaacgaagacgcaaccttcgtttacagtgtgaaccacgagtcctacgatcctgagaaccacaacgtgatctccggcgcatcttgcaccaccaactgcctcgcaccaatggcaaaggtcctgaacgacaagttcggcatcgagaacggcctcatgaccaccgttcacgcatacaccggcgaccagcgcctgcacgatgcacctcaccgcgacctgcgtcgtgcacgtgcagcagcagtcaacatcgttcctacctccaccggtgcagctaaggctgttgctctggttctcccagagctcaagggcaagcttgacggctacgcacttcgcgttccagttatcaccggttccgcaaccgacctgaccttcaacaccaagtctgaggtcaccgttgagtccatcaacgctgcaatcaaggaagctgcagtcggcgagttcggcgagaccctggcttactccgaagagccactggtttccaccgacatcgtccacgattcccacggctccatcttcgacgctggcctgaccaaggtctccggcaacaccgtcaaggttgtttcctggtacgacaacgagtggggctacacctgccagctcctgcgtctgaccgagctcgtagcttccaagctctaa

SEQ ID NO: 3 - protein, 334 aa, Artificial Sequence
  Wild-type glyceraldehyde-3-phosphate dehydrogenase
MTIRVGINGFGRIGRNFFRAVLERSDDLEVVAVNDLTDNKTLSTLLKFDSIMGRLGQEVEYDDDSITVGGKRIAVYAERDPKNLDWAAHNVDIVIESTGFFTDANAAKAHIEAGAKKVIISAPASNEDATFVYGVNHESYDPENHNVISGASCTTNCLAPMAKVLNDKFGIENGLMTTVHAYTGDQRLHDAPHRDLRRARAAAVNIVPTSTGAAKAVALVLPELKGKLDGYALRVPVITGSATDLTFNTKSEVTVESINAAIKEAAVGEFGETLAYSEEPLVSTDIVHDSHGSIFDAGLTKVSGNTVKVVSWYDNEWGYTCQLLRLTELVASKL

SEQ ID NO: 4 - DNA, 1005 bp, Artificial Sequence
  Wild-type glyceraldehyde-3-phosphate dehydrogenase coding gene
atgaccattcgtgttggtattaacggatttggccgtatcggacgtaacttcttccgcgcagttctagagcgcagcgacgatctcgaggtagttgcagtcaacgacctcaccgacaacaagaccctttccacccttctcaagttcgactccatcatgggccgccttggccaggaagttgaatacgacgatgactccatcaccgttggtggcaagcgcatcgctgtttacgcagagcgcgatccaaagaacctggactgggctgcacacaacgttgacatcgtgatcgagtccaccggcttcttcaccgatgcaaacgcggctaaggctcacatcgaagcaggtgccaagaaggtcatcatctccgcaccagcaagcaacgaagacgcaaccttcgtttacggtgtgaaccacgagtcctacgatcctgagaaccacaacgtgatctccggcgcatcttgcaccaccaactgcctcgcaccaatggcaaaggtcctgaacgacaagttcggcatcgagaacggcctcatgaccaccgttcacgcatacaccggcgaccagcgcctgcacgatgcacctcaccgcgacctgcgtcgtgcacgtgcagcagcagtcaacatcgttcctacctccaccggtgcagctaaggctgttgctctggttctcccagagctcaagggcaagcttgacggctacgcacttcgcgttccagttatcaccggttccgcaaccgacctgaccttcaacaccaagtctgaggtcaccgttgagtccatcaacgctgcaatcaaggaagctgcagtcggcgagttcggcgagaccctggcttactccgaagagccactggtttccaccgacatcgtccacgattcccacggctccatcttcgacgctggcctgaccaaggtctccggcaacaccgtcaaggttgtttcctggtacgacaacgagtggggctacacctgccagctcctgcgtctgaccgagctcgtagcttccaagctctaa

SEQ ID NO: 5 - DNA, 40 bp, Artificial Sequence
  gapA_1F
tgaattcgagctcggtacccttctgtcagctcaagaattc

SEQ ID NO: 6 - DNA, 33 bp, Artificial Sequence
  gapA_2R
gactcgtggttcacactgtaaacgaaggttgcg

SEQ ID NO: 7 - DNA, 33 bp, Artificial Sequence
  gapA_3F
cgcaaccttcgtttacagtgtgaaccacgagtc

SEQ ID NO: 8 - DNA, 40 bp, Artificial Sequence
  gapA_4R
gtcgactctagaggatccccaactaattagagcttggaag

SEQ ID NO: 9 - DNA, 20 bp, Artificial Sequence
  gapA_5F
ttctgtcagctcaagaattc

SEQ ID NO: 10 - DNA, 20 bp, Artificial Sequence
  gapA_6R
aactaattagagcttggaag